European Patent Specification EP 2 249 634 B1, published October 23, 2024. Title: AGRONOMICALLY ELITE LETTUCE WITH QUANTITATIVE BREMIA LACTUCA RESISTANCE. Applicant: Koorevaar, Gerard N. van der Laan, Hieronymus J. M. Weber, Rosa I. Application Unknown. The sequence listing filed with the application follows.

SEQUENCE LISTING (12 sequences)

SEQ ID NO: 1 - DNA, 19 bp, Artificial Sequence
  Synthetic primer
ggagttcagggcctctgtc

SEQ ID NO: 2 - DNA, 20 bp, Artificial Sequence
  Synthetic primer
ccgattctgcggttatcttc

SEQ ID NO: 3 - DNA, 20 bp, Artificial Sequence
  Synthetic primer
tttgggttccttcagtttgc

SEQ ID NO: 4 - DNA, 20 bp, Artificial Sequence
  Synthetic primer
cacagtttgggatgaacacg

SEQ ID NO: 5 - DNA, 20 bp, Artificial Sequence
  Synthetic primer
cggttgctcaagacctctca

SEQ ID NO: 6 - DNA, 19 bp, Artificial Sequence
  Synthetic primer
agcgaacgaccctctaacg

SEQ ID NO: 7 - DNA, 22 bp, Artificial Sequence
  Synthetic primer
ggaggttcatggcctactttac

SEQ ID NO: 8 - DNA, 21 bp, Artificial Sequence
  Synthetic primer
ggctcaatgactgacacttgc

SEQ ID NO: 9 - DNA, 20 bp, Artificial Sequence
  Synthetic primer
cgttgacaaccactcaccac

SEQ ID NO: 10 - DNA, 20 bp, Artificial Sequence
  Synthetic primer
actgaagtttttggcgaagc

SEQ ID NO: 11 - DNA, 20 bp, Artificial Sequence
  Synthetic primer
gaaaccagaggaggcagttg

SEQ ID NO: 12 - DNA, 22 bp, Artificial Sequence
  Synthetic primer
gtgctgcttcttacaaccaaac